European Patent Application EP 4 481 037 A1, published December 25, 2024. Title: Novel variant of ATP synthase and method for preparing L-aromatic amino acid using the same. Applicant: DAESANG CORPORATION. Application KR. The sequence listing filed with the application follows.

SEQUENCE LISTING (24 sequences)

SEQ ID NO: 1 - protein, 460 aa, synthetic construct
MATGKIVQVIGAVVDVEFPQDAVPRVYDALEVQNGNERLVLEVQQQLGGGIVRTIAMGSSDGLRRGLDVKDLEHPIEVPVGKATLGRIMNVLGEPVDMKGEIGEEERWAIHRAAPSYEELSNSQELLETGIKVIDLMCPFAKGGKVGLFGGAGVGKTVNMMELIRNIAIEHSGYSVFAGVGERTREGNDFYHEMTDSNVIDKVSLVYGQMNEPPGNRLRVALTGLTMAEKFRDESRDVLLFVDNIYRYTLAGTEVSALLGRMPSAVGYQPTLAEEMGVLQERITSTKTGSITSVQAVYVPADDLTDPSPATTFAHLDATVVLSRQIASLGIYPAVDPLDSTSRQLDPLVVGQEHYDTARGVQSILQRYQELKDIIAILGMDELSEEDKLVVARARKIQRFLSQPFFVAEVFTGSPGKYVSLKDTIRGFKGIMEGEYDHLPEQAFYMVGSIEEAVEKAKKL

SEQ ID NO: 2 - DNA, 703 bp, synthetic construct
  source 1..703: mol_type = other DNA
atggctactggaaagattgtccaggtaatcggcgccgtagttgacgtcgaattccctcaggatgccgtaccgcgcgtgtacgatgctcttgaggtgcaaaatggtaatgagcgtctggtgctggaagttcagcagcagctcggcggcggtatcgtacgtaccatcgcaatgggttcctccgacggtctgcgtcgcggtctggatgtaaaagacctcgaacacccgattgaagtcccggtaggtaaagcgactctgggccgtatcatgaacgtactgggtgaaccggtcgacatgaaaggcgagatcggtgaagaagagcgttgggcgattcaccgcgcagcaccttcctacgaagagctgtcaaactctcaggaactgctggaaaccggtatcaaagttatcgacctgatgtgtccgttcgctaagggcggtaaagttggtctgttcggtggtgcgggtgtaggtaaaaccgtaaacatgatggagctcattcgtaacatcgcgatcgagcactccggttactctgtgtttgcgggcgtaggtgaacgtactcgtgagggtaacgacttctaccacgaaatgaccgactccaacgttatcgacaaagtatccctggtgtatggccagatgaacgagccgccgggaaaccgtctgcgcgttgctctgaccggtctgaccatggctgagaaattccgtgacgaaa

SEQ ID NO: 3 - protein, 460 aa, Escherichia coli
MATGKIVQVIGAVVDVEFPQDAVPRVYDALEVQNGNERLVLEVQQQLGGGIVRTIAMGSSDGLRRGLDVKDLEHPIEVPVGKATLGRIMNVLGEPVDMKGEIGEEERWAIHRAAPSYEELSNSQELLETGIKVIDLMCPFAKGGKVGLFGGAGVGKTVNMMELIRNIAIEHSGYSVFAGVGERTREGNDFYHEMTDSNVIDKVSLVYGQMNEPPGNRLRVALTGLTMAEKFRDEGRDVLLFVDNIYRYTLAGTEVSALLGRMPSAVGYQPTLAEEMGVLQERITSTKTGSITSVQAVYVPADDLTDPSPATTFAHLDATVVLSRQIASLGIYPAVDPLDSTSRQLDPLVVGQEHYDTARGVQSILQRYQELKDIIAILGMDELSEEDKLVVARARKIQRFLSQPFFVAEVFTGSPGKYVSLKDTIRGFKGIMEGEYDHLPEQAFYMVGSIEEAVEKAKKL

SEQ ID NO: 4 - DNA, 1383 bp, Escherichia coli
  source 1..1383: mol_type = genomic DNA
atggctactggaaagattgtccaggtaatcggcgccgtagttgacgtcgaattccctcaggatgccgtaccgcgcgtgtacgatgctcttgaggtgcaaaatggtaatgagcgtctggtgctggaagttcagcagcagctcggcggcggtatcgtacgtaccatcgcaatgggttcctccgacggtctgcgtcgcggtctggatgtaaaagacctcgaacacccgattgaagtcccggtaggtaaagcgactctgggccgtatcatgaacgtactgggtgaaccggtcgacatgaaaggcgagatcggtgaagaagagcgttgggcgattcaccgcgcagcaccttcctacgaagagctgtcaaactctcaggaactgctggaaaccggtatcaaagttatcgacctgatgtgtccgttcgctaagggcggtaaagttggtctgttcggtggtgcgggtgtaggtaaaaccgtaaacatgatggagctcattcgtaacatcgcgatcgagcactccggttactctgtgtttgcgggcgtaggtgaacgtactcgtgagggtaacgacttctaccacgaaatgaccgactccaacgttatcgacaaagtatccctggtgtatggccagatgaacgagccgccgggaaaccgtctgcgcgttgctctgaccggtctgaccatggctgagaaattccgtgacgaaggtcgtgacgttctgctgttcgttgacaacatctatcgttacaccctggccggtacggaagtatccgcactgctgggccgtatgccttcagcggtaggttatcagccgaccctggcggaagagatgggcgttctgcaggaacgtatcacctccaccaaaactggttctatcacctccgtacaggcagtatacgtacctgcggatgacttgactgacccgtctccggcaaccacctttgcgcaccttgacgcaaccgtggtactgagccgtcagatcgcgtctctgggtatctacccggccgttgacccgctggactccaccagccgtcagctggacccgctggtggttggtcaggaacactacgacaccgcgcgtggcgttcagtccatcctgcaacgttatcaggaactgaaagacatcatcgccatcctgggtatggatgaactgtctgaagaagacaaactggtggtagcgcgtgctcgtaagatccagcgcttcctgtcccagccgttcttcgtggcagaagtattcaccggttctccgggtaaatacgtctccctgaaagacaccatccgtggctttaaaggcatcatggaaggcgaatacgatcacctgccggagcaggcgttctacatggtcggttccatcgaagaagctgtggaaaaagccaaaaaactttaa

SEQ ID NO: 5 - DNA, 30 bp, synthetic construct
  source 1..30: mol_type = other DNA
caattttattatagtaattgactattatac

SEQ ID NO: 6 - DNA, 40 bp, synthetic construct
  source 1..40: mol_type = other DNA
cgtgacgttccaattttattatagtaattgactattatac

SEQ ID NO: 7 - DNA, 40 bp, synthetic construct
  source 1..40: mol_type = other DNA
gaacgtcacgaccttcgtcagttttagagctagaaatagc

SEQ ID NO: 8 - DNA, 30 bp, synthetic construct
  source 1..30: mol_type = other DNA
accttcgtcagttttagagctagaaatagc

SEQ ID NO: 9 - DNA, 21 bp, synthetic construct
  source 1..21: mol_type = other DNA
gagcctgtcggcctacctgct

SEQ ID NO: 10 - DNA, 20 bp, synthetic construct
  source 1..20: mol_type = other DNA
cggccggcatgagcctgtcg

SEQ ID NO: 11 - DNA, 31 bp, synthetic construct
  source 1..31: mol_type = other DNA
atgccggccgcggccgggtagatacccagag

SEQ ID NO: 12 - DNA, 21 bp, synthetic construct
  source 1..21: mol_type = other DNA
cggccgggtagatacccagag

SEQ ID NO: 13 - DNA, 20 bp, synthetic construct
  source 1..20: mol_type = other DNA
tctgctgttcgttgacaaca

SEQ ID NO: 14 - DNA, 20 bp, synthetic construct
  source 1..20: mol_type = other DNA
gtcgtgacgttctgctgttc

SEQ ID NO: 15 - DNA, 30 bp, synthetic construct
  source 1..30: mol_type = other DNA
acgtcacgactttcgtcacggaatttctca

SEQ ID NO: 16 - DNA, 20 bp, synthetic construct
  source 1..20: mol_type = other DNA
tttcgtcacggaatttctca

SEQ ID NO: 17 - DNA, 20 bp, synthetic construct
  source 1..20: mol_type = other DNA
tccgttcgctaagggcggta

SEQ ID NO: 18 - DNA, 20 bp, synthetic construct
  source 1..20: mol_type = other DNA
acctgatgtgtccgttcgct

SEQ ID NO: 19 - DNA, 33 bp, synthetic construct
  source 1..33: mol_type = other DNA
cacatcaggtgagctcctgaaaatctcgataac

SEQ ID NO: 20 - DNA, 23 bp, synthetic construct
  source 1..23: mol_type = other DNA
gagctcctgaaaatctcgataac

SEQ ID NO: 21 - DNA, 20 bp, synthetic construct
  source 1..20: mol_type = other DNA
tccgttcgctaagggcggta

SEQ ID NO: 22 - DNA, 20 bp, synthetic construct
  source 1..20: mol_type = other DNA
acctgatgtgtccgttcgct

SEQ ID NO: 23 - DNA, 3234 bp, synthetic construct
  source 1..3234: mol_type = other DNA
tttccataggctccgcccccctgacgagcatcacaaaaatcgacgctcaagtcagaggtggcgaaacccgacaggactataaagataccaggcgtttccccctggaagctccctcgtgcgctctcctgttccgaccctgccgcttaccggatacctgtccgcctttctcccttcgggaagcgtggcgctttctcatagctcacgctgtaggtatctcagttcggtgtaggtcgttcgctccaagctgggctgtgtgcacgaaccccccgttcagcccgaccgctgcgccttatccggtaactatcgtcttgagtccaacccggtaagacacgacttatcgccactggcagcagccactggtaacaggattagcagagcgaggtatgtaggcggtgctacagagttcttgaagtggtggcctaactacggctacactagaaggacagtatttggtatctgcgctctgctgaagccagttaccttcggaaaaagagttggtagctcttgatccggcaaacaaaccaccgctggtagcggtggtttttttgtttgcaagcagcagattacgcgcagaaaaaaaggatctcaagaagatcctttgatcttttctacggggtctgacgctcagtggaacgaaaactcacgttaagggattttggtcatgagattatcaaaaaggatcttcacctagatccttttaaattaaaaatgaagttttaaatcaatctaaagtatatatgagtaaacttggtctgacagttaaaagattgacagtataatagtcaattactataataaaattgatgcgcaggtgaaacacctgctgcagttttagagctagaaatagcaagttaaaataaggctagtccgttatcaacttgaaaaagtggcaccgagtcggtgctttttttcgttttccgggacgccctcgcggacgtgctcatagtccacgacgcccgtgattttgtagccctggccgacggccagcaggtaggccgacaggctcatgccggccggagctcctgaaaatctcgataactcaaaaaatacgcccggtagtgatcttatttcattatggtgaaagttggaacctcttaggatcctctagatttaagaaggagatatacataaaactccttctgagctagttctctagcattctattattttgattcgacaccttaataatagcagaaggagtttttacctgtcaaagaaccatcaaacccttgatacacaaggctttgacctaattttgaaaaatgatgttgtttctatatagtatcaagataagaaagaaaaggatttttcgctacgctcaaatcctttcccgtcacgggcttctcagggcgttttatggcgggtctgctatgtggtgctatctgactttttgctgttcagcagttcctgccctctgattttccagtctgaccacttcggattatcccgtgacaggtcattcagactggctaatgcacccagtaaggcagcggtatcatcaacggggtctgacgctcagtggaacgaaaactcacgttaagggattttggtcatgagattatcaaaaaggatcttcacctagatccttttaaattaaaaatgaagttttaaatcaatctaaagtatatatgagtaaacttggtctgacagttaccaatgcttaatcagtgaggcacctatctcagcgatctgtctatttcgttcatccatagttgcctgactccccgtcgtgtagataactacgatacgggagggcttaccatctggccccagtgctgcaatgataccgcgagacccacgctcaccggctccagatttatcagcaataaaccagccagccggaagggccgagcgcagaagtggtcctgcaactttatccgcctccatccagtctattaattgttgccgggaagctagagtaagtagttcgccagttaatagtttgcgcaacgttgttgccattgctacaggcatcgtggtgtcacgctcgtcgtttggtatggcttcattcagctccggttcccaacgatcaaggcgagttacatgatcccccatgttgtgcaaaaaagcggttagctccttcggtcctccgatcgttgtcagaagtaagttggccgcagtgttatcactcatggttatggcagcactgcataattctcttactgtcatgccatccgtaagatgcttttctgtgactggtgagtactcaaccaagtcattctgagaatagtgtatgcggcgaccgagttgctcttgcccggcgtcaatacgggataataccgcgccacatagcagaactttaaaagtgctcatcattggaaaacgttcttcggggcgaaaactctcaaggatcttaccgctgttgagatccagttcgatgtaacccactcgtgcacccaactgatcttcagcatcttttactttcaccagcgtttctgggtgagcaaaaacaggaaggcaaaatgccgcaaaaaagggaataagggcgacacggaaatgttgaatactcatactcttcctttttcaatattattgaagcatttatcagggttattgtctcatgagcggatacatatttgaatgtatttagaaaaataaacaaataggggttccgcgcacatttccccgaaaagtgccaccaaaaaaacacaaaagaccacattttttaatgtggtctttattcttcaactaaagcacccattagttcaacaaacgaaaattggataaagtgggatatttttaaaatatatatttatgttacagtaagctgcctcgcgcgtttcggtgatgacggtgaaaacctctgacacatgcagctcccggagacggtcacagcttgtctgtaagcggatgccgggagcagacaagcccgtcagggcgcgtcagcgggtgttggcgggtgtcggggcgcagccatgacccagtcacgtagcgatagcggagtgtatactggcttaactatgcggcatcagagcagattgtactgagagtgcaccatatgcggtgtgaaataccgcacagatgcgtaaggagaaaataccgcatcaggcgctcttccgcttcctcgctcactgactcgctgcgctcggtcgttcggctgcggcgagcggtatcagctcactcaaaggcggtaatacggttatccacagaatcaggggataacgcaggaaagaacatgtgagcaaaaggccagcaaaaggccaggaaccgtaaaaaggccgcgttgctggcgtt

SEQ ID NO: 24 - DNA, 9656 bp, synthetic construct
  source 1..9656: mol_type = other DNA
aaagccatgacaaaaacgcgtaacaaaagtgtctataatcacggcagaaaagtccacattgattatttgcacggcgtcacactttgctatgccatagcatttttatccataagattagcggatcctacctgacgctttttatcgcaactctctactgtttctccatacccgtttttttgggaattcgagctctaaggaggttataaaaaatggatattaatactgaaactgagatcaagcaaaagcattcactaaccccctttcctgttttcctaatcagcccggcatttcgcgggcgatattttcacagctatttcaggagttcagccatgaacgcttattacattcaggatcgtcttgaggctcagagctgggcgcgtcactaccagcagctcgcccgtgaagagaaagaggcagaactggcagacgacatggaaaaaggcctgccccagcacctgtttgaatcgctatgcatcgatcatttgcaacgccacggggccagcaaaaaatccattacccgtgcgtttgatgacgatgttgagtttcaggagcgcatggcagaacacatccggtacatggttgaaaccattgctcaccaccaggttgatattgattcagaggtataaaacgaatgagtactgcactcgcaacgctggctgggaagctggctgaacgtgtcggcatggattctgtcgacccacaggaactgatcaccactcttcgccagacggcatttaaaggtgatgccagcgatgcgcagttcatcgcattactgatcgttgccaaccagtacggccttaatccgtggacgaaagaaatttacgcctttcctgataagcagaatggcatcgttccggtggtgggcgttgatggctggtcccgcatcatcaatgaaaaccagcagtttgatggcatggactttgagcaggacaatgaatcctgtacatgccggatttaccgcaaggaccgtaatcatccgatctgcgttaccgaatggatggatgaatgccgccgcgaaccattcaaaactcgcgaaggcagagaaatcacggggccgtggcagtcgcatcccaaacggatgttacgtcataaagccatgattcagtgtgcccgtctggccttcggatttgctggtatctatgacaaggatgaagccgagcgcattgtcgaaaatactgcatacactgcagaacgtcagccggaacgcgacatcactccggttaacgatgaaaccatgcaggagattaacactctgctgatcgccctggataaaacatgggatgacgacttattgccgctctgttcccagatatttcgccgcgacattcgtgcatcgtcagaactgacacaggccgaagcagtaaaagctcttggattcctgaaacagaaagccgcagagcagaaggtggcagcatgacaccggacattatcctgcagcgtaccgggatcgatgtgagagctgtcgaacagggggatgatgcgtggcacaaattacggctcggcgtcatcaccgcttcagaagttcacaacgtgatagcaaaaccccgctccggaaagaagtggcctgacatgaaaatgtcctacttccacaccctgcttgctgaggtttgcaccggtgtggctccggaagttaacgctaaagcactggcctggggaaaacagtacgagaacgacgccagaaccctgtttgaattcacttccggcgtgaatgttactgaatccccgatcatctatcgcgacgaaagtatgcgtaccgcctgctctcccgatggtttatgcagtgacggcaacggccttgaactgaaatgcccgtttacctcccgggatttcatgaagttccggctcggtggtttcgaggccataaagtcagcttacatggcccaggtgcagtacagcatgtgggtgacgcgaaaaaatgcctggtactttgccaactatgacccgcgtatgaagcgtgaaggcctgcattatgtcgtgattgagcgggatgaaaagtacatggcgagttttgacgagatcgtgccggagttcatcgaaaaaatggacgaggcactggctgaaattggttttgtatttggggagcaatggcgatgagatctaaagaggagaaaggatctatggataagaaatactcaataggcttagatatcggcacaaatagcgtcggatgggcggtgatcactgatgaatataaggttccgtctaaaaagttcaaggttctgggaaatacagaccgccacagtatcaaaaaaaatcttataggggctcttttatttgacagtggagagacagcggaagcgactcgtctcaaacggacagctcgtagaaggtatacacgtcggaagaatcgtatttgttatctacaggagattttttcaaatgagatggcgaaagtagatgatagtttctttcatcgacttgaagagtcttttttggtggaagaagacaagaagcatgaacgtcatcctatttttggaaatatagtagatgaagttgcttatcatgagaaatatccaactatctatcatctgcgaaaaaaattggtagattctactgataaagcggatttgcgcttaatctatttggccttagcgcatatgattaagtttcgtggtcattttttgattgagggagatttaaatcctgataatagtgatgtggacaaactatttatccagttggtacaaacctacaatcaattatttgaagaaaaccctattaacgcaagtggagtagatgctaaagcgattctttctgcacgattgagtaaatcaagacgattagaaaatctcattgctcagctccccggtgagaagaaaaatggcttatttgggaatctcattgctttgtcattgggtttgacccctaattttaaatcaaattttgatttggcagaagatgctaaattacagctttcaaaagatacttacgatgatgatttagataatttattggcgcaaattggagatcaatatgctgatttgtttttggcagctaagaatttatcagatgctattttactttcagatatcctaagagtaaatactgaaataactaaggctcccctatcagcttcaatgattaaacgctacgatgaacatcatcaagacttgactcttttaaaagctttagttcgacaacaacttccagaaaagtataaagaaatcttttttgatcaatcaaaaaacggatatgcaggttatattgatgggggagctagccaagaagaattttataaatttatcaaaccaattttagaaaaaatggatggtactgaggaattattggtgaaactaaatcgtgaagatttgctgcgcaagcaacggacctttgacaacggctctattccccatcaaattcacttgggtgagctgcatgctattttgagaagacaagaagacttttatccatttttaaaagacaatcgtgagaagattgaaaaaatcttgacttttcgaattccttattatgttggtccattggcgcgtggcaatagtcgttttgcatggatgactcggaagtctgaagaaacaattaccccatggaattttgaagaagttgtcgataaaggtgcttcagctcaatcatttattgaacgcatgacaaactttgataaaaatcttccaaatgaaaaagtactaccaaaacatagtttgctttatgagtattttacggtttataacgaattgacaaaggtcaaatatgttactgaaggaatgcgaaaaccagcatttctttcaggtgaacagaagaaagccattgttgatttactcttcaaaacaaatcgaaaagtaaccgttaagcaattaaaagaagattatttcaaaaaaatagaatgttttgatagtgttgaaatttcaggagttgaagatagatttaatgcttcattaggtacctaccatgatttgctaaaaattattaaagataaagattttttggataatgaagaaaatgaagatatcttagaggatattgttttaacattgaccttatttgaagatagggagatgattgaggaaagacttaaaacatatgctcacctctttgatgataaggtgatgaaacagcttaaacgtcgccgttatactggttggggacgtttgtctcgaaaattgattaatggtattagggataagcaatctggcaaaacaatattagattttttgaaatcagatggttttgccaatcgcaattttatgcagctgatccatgatgatagtttgacatttaaagaagacattcaaaaagcacaagtgtctggacaaggcgatagtttacatgaacatattgcaaatttagctggtagccctgctattaaaaaaggtattttacagactgtaaaagttgttgatgaattggtcaaagtaatggggcggcataagccagaaaatatcgttattgaaatggcacgtgaaaatcagacaactcaaaagggccagaaaaattcgcgagagcgtatgaaacgaatcgaagaaggtatcaaagaattaggaagtcagattcttaaagagcatcctgttgaaaatactcaattgcaaaatgaaaagctctatctctattatctccaaaatggaagagacatgtatgtggaccaagaattagatattaatcgtttaagtgattatgatgtcgatcacattgttccacaaagtttccttaaagacgattcaatagacaataaggtcttaacgcgttctgataaaaatcgtggtaaatcggataacgttccaagtgaagaagtagtcaaaaagatgaaaaactattggagacaacttctaaacgccaagttaatcactcaacgtaagtttgataatttaacgaaagctgaacgtggaggtttgagtgaacttgataaagctggttttatcaaacgccaattggttgaaactcgccaaatcactaagcatgtggcacaaattttggatagtcgcatgaatactaaatacgatgaaaatgataaacttattcgagaggttaaagtgattaccttaaaatctaaattagtttctgacttccgaaaagatttccaattctataaagtacgtgagattaacaattaccatcatgcccatgatgcgtatctaaatgccgtcgttggaactgctttgattaagaaatatccaaaacttgaatcggagtttgtctatggtgattataaagtttatgatgttcgtaaaatgattgctaagtctgagcaagaaataggcaaagcaaccgcaaaatatttcttttactctaatatcatgaacttcttcaaaacagaaattacacttgcaaatggagagattcgcaaacgccctctaatcgaaactaatggggaaactggagaaattgtctgggataaagggcgagattttgccacagtgcgcaaagtattgtccatgccccaagtcaatattgtcaagaaaacagaagtacagacaggcggattctccaaggagtcaattttaccaaaaagaaattcggacaagcttattgctcgtaaaaaagactgggatccaaaaaaatatggtggttttgatagtccaacggtagcttattcagtcctagtggttgctaaggtggaaaaagggaaatcgaagaagttaaaatccgttaaagagttactagggatcacaattatggaaagaagttcctttgaaaaaaatccgattgactttttagaagctaaaggatataaggaagttaaaaaagacttaatcattaaactacctaaatatagtctttttgagttagaaaacggtcgtaaacggatgctggctagtgccggagaattacaaaaaggaaatgagctggctctgccaagcaaatatgtgaattttttatatttagctagtcattatgaaaagttgaagggtagtccagaagataacgaacaaaaacaattgtttgtggagcagcataagcattatttagatgagattattgagcaaatcagtgaattttctaagcgtgttattttagcagatgccaatttagataaagttcttagtgcatataacaaacatagagacaaaccaatacgtgaacaagcagaaaatattattcatttatttacgttgacgaatcttggagctcccgctgcttttaaatattttgatacaacaattgatcgtaaacgatatacgtctacaaaagaagttttagatgccactcttatccatcaatccatcactggtctttatgaaacacgcattgatttgagtcagctaggaggtgactaacgcatcctcacgataatatccgggtaggcgcaatcactttcgtctactccgttacaaagcgaggctgggtatttcccggcctttctgttatccgaaatccactgaaagcacagcggctggctgaggagataaataataaacgaggggctgtatgcacaaagcatcttctgttgagttaagaacgagtatcgagatggcacatagccttgctcaaattggaatcaggtttgtgccaataccagtagaaacagacgaagaatccatgggtatggacagttttccctttgatatgtaacggtgaacagttgttctacttttgtttgttagtcttgatgcttcactgatagatacaagagccaaatctagtaatattttatctgattaataagatgatcttcttgagatcgttttggtctgcgcgtaatctcttgctctgaaaacgaaaaaaccgccttgcagggcggtttttcgaaggttctctgagctaccaactctttgaaccgaggtaactggcttggaggagcgcagtcaccaaaacttgtcctttcagtttagccttaaccggcgcatgacttcaagactaactcctctaaatcaattaccagtggctgctgccagtggtgcttttgcatgtctttccgggttggactcaagacgatagttaccggataaggcgcagcggtcggactgaacggggggttcgtgcatacagtccagcttggagcgaactgcctacccggaactgagtgtcaggcgtggaatgagacaaacgcggccataacagcggaatgacaccggtaaaccgaaaggcaggaacaggagagcgcacgagggagccgccagggggaaacgcctggtatctttatagtcctgtcgggtttcgccaccactgatttgagcgtcagatttcgtgatgcttgtcaggggggcggagcctatggaaaaacggctttgccgcggccccgctgaatattccttttgtctccgaccatcaggcacctgagtcgctgtctttttcgtgacattcagttcgctgcgctcacggctctggcagtgaatgggggtaaatggcactacaggcgccttttatggattcatgcaaggaaactacccataatacaagaaaagatgtggtctttattcttcaactaaagcacccattagttcaacaaacgaaaattggataaagtgggatatttttaaaatatatatttatgttacctggcagagcctgtactttttacagtcggttttctaatgtcactaacctgccccgttagtcgccatttgcatcgatttattatgacaacttgacggctacatcattcactttttcttcacaaccggcacggaactcgctcgggctggccccggtgcattttttaaatacccgcgagaaatagagttgatcgtcaaaaccaacattgcgaccgacggtggcgataggcatccgggtggtgctcaaaagcagcttcgcctggctgatacgttggtcctcgcgccagcttaagacgctaatccctaactgctggcggaaaagatgtgacagacgcgacggcgacaagcaaacatgctgtgcgacgctggcgatatcaaaattgctgtctgccaggtgatcgctgatgtactgacaagcctcgcgtacccgattatccatcggtggatggagcgactcgttaatcgcttccatgcgccgcagtaacaattgctcaagcagatttatcgccagcagctccgaatagcgcccttccccttgcccggcgttaatgatttgcccaaacaggtcgctgaaatgcggctggtgcgcttcatccgggcgaaagaaccccgtattggcaaatattgacggccagttaagccattcatgccagtaggcgcgcggacgaaagtaaacccactggtgataccattcgcgagcctccggatgacgaccgtagtgatgaatctctcctggcgggaacagcaaaatatcacccggtcggcaaacaaattctcgtccctgatttttcaccaccccctgaccgcgaatggtgagattgagaatataacctttcattcccagcggtcggtcgataaaaaaatcgagataaccgttggcctcaatcggcgttaaacccgccaccagatgggcattaaacgagtatcccggcagcaggggatcattttgcgcttcagccatacttttcatactcccgccattcagagaagaaaccaattgtccatattgcatcagacattgccgtcactgcgtcttttactggctcttctcgctaaccaaaccggtaaccccgcttattaaaagcattctgtaacaaagcgggaccagtaatagaaagtgagggagccacggttgatgagagctttgttgtaggtggaccagttggtgattttgaacttttgctttgccacggaacggtctgcgttgtcgggaagatgcgtgatctgatccttcaactcagcaaaagttcgatttattcaacaaagccacgttgtgtctcaaaatctctgatgttacattgcacaagataaaaatatatcatcatgaacaataaaactgtctgcttacataaacagtaatacaaggggtgttatgagccatattcaacgggaaacgtcttgctcgaggccgcgattaaattccaacatggatgctgatttatatgggtataaatgggctcgcgataatgtcgggcaatcaggtgcgacaatctatcgattgtatgggaagcccgatgcgccagagttgtttctgaaacatggcaaaggtagcgttgccaatgatgttacagatgagatggtcagactaaactggctgacggaatttatgcctcttccgaccatcaagcattttatccgtactcctgatgatgcatggttactcaccactgcgatccccgggaaaacagcattccaggtattagaagaatatcctgattcaggtgaaaatattgttgatgcgctggcagtgttcctgcgccggttgcattcgattcctgtttgtaattgtccttttaacagcgatcgcgtatttcgtctcgctcaggcgcaatcacgaatgaataacggtttggttgatgcgagtgattttgatgacgagcgtaatggctggcctgttgaacaagtctggaaagaaatgcataagcttttgccattctcaccggattcagtcgtcactcatggtgatttctcacttgataaccttatttttgacgaggggaaattaataggttgtattgatgttggacgagtcggaatcgcagaccgataccaggatcttgccatcctatggaactgcctcggtgagttttctccttcattacagaaacggctttttcaaaaatatggtattgataatcctgatatgaataaattgcagtttcatttgatgctcgatgagtttttctaatcagaattggttaattggttgtaaca